European Patent Application EP 4 169 532 A1, published April 26, 2023. Title: Molecular targeted drug and companion diagnostic drug. Applicant: National University Corporation Tokai National Higher Education and Research System. The sequence listing filed with the application follows.

SEQUENCE LISTING (12 sequences)

SEQ ID NO: 1 - DNA, 18 bp, synthetic construct
  misc_feature 1..18: note = PCR primer
  source 1..18: mol_type = other DNA
agcgaggacgatgaccag

SEQ ID NO: 2 - DNA, 20 bp, synthetic construct
  misc_feature 1..20: note = PCR primer
  source 1..20: mol_type = other DNA
ggtgccaaagacacagacaa

SEQ ID NO: 3 - DNA, 20 bp, synthetic construct
  misc_feature 1..20: note = PCR primer
  source 1..20: mol_type = other DNA
tcattctggagctggaggac

SEQ ID NO: 4 - DNA, 19 bp, synthetic construct
  misc_feature 1..19: note = PCR primer
  source 1..19: mol_type = other DNA
ggcagctgagaggttcaca

SEQ ID NO: 5 - DNA, 19 bp, synthetic construct
  misc_feature 1..19: note = PCR primer
  source 1..19: mol_type = other DNA
gaaggtgaaggtcggagtc

SEQ ID NO: 6 - DNA, 20 bp, synthetic construct
  misc_feature 1..20: note = PCR primer
  source 1..20: mol_type = other DNA
gaagatggtgatgggatttc

SEQ ID NO: 7 - DNA, 20 bp, synthetic construct
  misc_feature 1..20: note = PCR primer
  source 1..20: mol_type = other DNA
caagcttcccgttctcagcc

SEQ ID NO: 8 - protein, 18 aa, synthetic construct
  REGION 1..18: note = CHRNB2_#94-111
WKPEEFDNMKKVRLPSKH

SEQ ID NO: 9 - protein, 13 aa, synthetic construct
  REGION 1..13: note = CHRNB2_#490-502
TFLHSDHSAPSSK

SEQ ID NO: 10 - protein, 18 aa, synthetic construct
  REGION 1..18: note = NPTXR_#161-178
CESGLPRGLQGAGPRRDT

SEQ ID NO: 11 - protein, 18 aa, synthetic construct
  REGION 1..18: note = NPTXR_#251-268
KERVALSHSSRRQRQEVE

SEQ ID NO: 12 - protein, 15 aa, synthetic construct
  REGION 1..15: note = NH-01 epitope
GLPRGLQGAGPRRDT